European Patent Application EP 4 591 879 A2, published July 30, 2025. Title: MULTISPECIFIC ANTIBODIES HAVING SPECIFICITY FOR TNFa AND IL-17A, ANTIBODIES TARGETING IL-17A, AND METHODS OF USE THEREOF. Applicant: Numab Therapeutics AG. Application WO PCT/EP2020/052481, filed January 31, 2020. The sequence listing filed with the application follows.

SEQUENCE LISTING (149 sequences)

SEQ ID NO: 1 - protein, 11 aa, synthetic construct
  REGION 1..11: note = artificial antibody-related sequence
GFSFSSDYWMC

SEQ ID NO: 2 - protein, 18 aa, synthetic construct
  REGION 1..18: note = artificial antibody-related sequence
CIYAGDVDDTDYASWARG

SEQ ID NO: 3 - protein, 12 aa, synthetic construct
  REGION 1..12: note = artificial antibody-related sequence
RVDGFDITYFDL

SEQ ID NO: 4 - protein, 6 aa, synthetic construct
  REGION 1..6: note = artificial antibody-related sequence
SDYWMC

SEQ ID NO: 5 - protein, 18 aa, synthetic construct
  REGION 1..18: note = artificial antibody-related sequence
CIYAGDVDDTDYASWARG

SEQ ID NO: 6 - protein, 11 aa, synthetic construct
  REGION 1..11: note = artificial antibody-related sequence
VDGFDITYFDL

SEQ ID NO: 7 - protein, 8 aa, synthetic construct
  REGION 1..8: note = artificial antibody-related sequence
GFSFSSDY

SEQ ID NO: 8 - protein, 5 aa, synthetic construct
  REGION 1..5: note = artificial antibody-related sequence
AGDVD

SEQ ID NO: 9 - protein, 9 aa, synthetic construct
  REGION 1..9: note = artificial antibody-related sequence
DGFDITYFD

SEQ ID NO: 10 - protein, 122 aa, synthetic construct
  REGION 1..122: note = artificial antibody-related sequence
EVQLVESGGGLVQPGGSLRLSCAASGFSFSSDYWMCWVRQAPGKGLEWIGCIYAGDVDDTDYASWARGRFTISRDNSKNTVYLQMNSLRAEDTAVYYCARVDGFDITYFDLWGQGTLVTVSS

SEQ ID NO: 11 - protein, 122 aa, synthetic construct
  REGION 1..122: note = artificial antibody-related sequence
EVQLVESGGGLVKPEGSLRLSCAASGFSFSSDYWMCWVRQAPGKGLEWIACIYAGDVDDTDYASWARGRFTISRDNSKNTVYLQMNSLRAEDTAVYYCARVDGFDITYFDLWGQGTLVTVSS

SEQ ID NO: 12 - protein, 11 aa, synthetic construct
  REGION 1..11: note = artificial antibody-related sequence
QASQTINYWLA

SEQ ID NO: 13 - protein, 7 aa, synthetic construct
  REGION 1..7: note = artificial antibody-related sequence
RASTLAS

SEQ ID NO: 14 - protein, 12 aa, synthetic construct
  REGION 1..12: note = artificial antibody-related sequence
QNYYYSTSRSYG

SEQ ID NO: 15 - protein, 11 aa, synthetic construct
  REGION 1..11: note = artificial antibody-related sequence
QASQTINYWLA

SEQ ID NO: 16 - protein, 7 aa, synthetic construct
  REGION 1..7: note = artificial antibody-related sequence
RASTLAS

SEQ ID NO: 17 - protein, 12 aa, synthetic construct
  REGION 1..12: note = artificial antibody-related sequence
QNYYYSTSRSYG

SEQ ID NO: 18 - protein, 7 aa, synthetic construct
  REGION 1..7: note = artificial antibody-related sequence
SQTINYW

SEQ ID NO: 19 - skipped

SEQ ID NO: 20 - protein, 9 aa, synthetic construct
  REGION 1..9: note = artificial antibody-related sequence
YYYSTSRSY

SEQ ID NO: 21 - protein, 111 aa, synthetic construct
  REGION 1..111: note = artificial antibody-related sequence
DIQMTQSPSSLSASVGDRVTITCQASQTINYWLAWYQQKPGKAPKLLIYRASTLASGVPSRFSGSGSGTDFTLTISSLQPEDFATYYCQNYYYSTSRSYGFGGGTKLTVLG

SEQ ID NO: 22 - protein, 111 aa, synthetic construct
  REGION 1..111: note = artificial antibody-related sequence
DIQMTQSPSSLSASVGDRVTITCQASQTINYWLAWYQQKPGKPPKLLIYRASTLASGVPSRFSGSGSGTDFTLTISSLQPEDFATYYCQNYYYSTSRSYGFGGGTKLTVLG

SEQ ID NO: 23 - protein, 20 aa, synthetic construct
  REGION 1..20: note = artificial antibody-related sequence
GGGGSGGGGSGGGGSGGGGS

SEQ ID NO: 24 - protein, 253 aa, synthetic construct
  REGION 1..253: note = artificial antibody-related sequence
DIQMTQSPSSLSASVGDRVTITCQASQTINYWLAWYQQKPGKAPKLLIYRASTLASGVPSRFSGSGSGTDFTLTISSLQPEDFATYYCQNYYYSTSRSYGFGGGTKLTVLGGGGGSGGGGSGGGGSGGGGSEVQLVESGGGLVQPGGSLRLSCAASGFSFSSDYWMCWVRQAPGKGLEWIGCIYAGDVDDTDYASWARGRFTISRDNSKNTVYLQMNSLRAEDTAVYYCARVDGFDITYFDLWGQGTLVTVSS

SEQ ID NO: 25 - protein, 253 aa, synthetic construct
  REGION 1..253: note = artificial antibody-related sequence
DIQMTQSPSSLSASVGDRVTITCQASQTINYWLAWYQQKPGKPPKLLIYRASTLASGVPSRFSGSGSGTDFTLTISSLQPEDFATYYCQNYYYSTSRSYGFGGGTKLTVLGGGGGSGGGGSGGGGSGGGGSEVQLVESGGGLVKPEGSLRLSCAASGFSFSSDYWMCWVRQAPGKGLEWIACIYAGDVDDTDYASWARGRFTISRDNSKNTVYLQMNSLRAEDTAVYYCARVDGFDITYFDLWGQGTLVTVSS

SEQ ID NO: 26 - protein, 11 aa, Homo sapiens
FGTGTKVTVLG

SEQ ID NO: 27 - protein, 11 aa, Homo sapiens
FGGGTKLTVLG

SEQ ID NO: 28 - protein, 11 aa, Homo sapiens
FGGGTQLIILG

SEQ ID NO: 29 - protein, 11 aa, Homo sapiens
FGEGTELTVLG

SEQ ID NO: 30 - protein, 11 aa, Homo sapiens
FGSGTKVTVLG

SEQ ID NO: 31 - protein, 11 aa, Homo sapiens
FGGGTQLTVLG

SEQ ID NO: 32 - protein, 11 aa, Homo sapiens
FGGGTQLTALG

SEQ ID NO: 33 - protein, 155 aa, Homo sapiens
MTPGKTSLVSLLLLLSLEAIVKAGIAIPQNPGCPNSEDKNFPRTVMVNLNIHNRNTNTNPKRSSDYYNRSTSPWNLHRNEDPERYPSVIWEAKCRHLGCVNADGKVDYHMNSVPIQQEILVLRREPPHCPNSFRLEKILVSVGCTCVTPIVHHVS

SEQ ID NO: 34 - protein, 180 aa, Homo sapiens
MDWPHNLLFLLTISIFLGLGQPRSPKSKRKGQGRPGPLAPGPHQVPLDLVSRMKPYARMEEYERNIEEMVAQLRNSSELAQRKCEVNLQLWMSNKRSLSPWGYSINHDPSRIPVDLPEARCLCLGCVNPFTMQEDRSMVSVPVFSQVPVRRRLCPPPPRTGPCRQRAVMETIAVGCTCIF

SEQ ID NO: 35 - protein, 197 aa, Homo sapiens
MTLLPGLLFLTWLHTCLAHHDPSLRGHPHSHGTPHCYSAEELPLGQAPPHLLARGAKWGQALPVALVSSLEAASHRGRHERPSATTQCPVLRPEEVLEADTHQRSISPWRYRVDTDEDRYPQKLAFAECLCRGCIDARTGRETAALNSVRLLQSLLVLRRRPCSRDGSGLPTPGAFAFHTEFIHVPVGCTCVLPRSV

SEQ ID NO: 36 - protein, 202 aa, Homo sapiens
MLVAGFLLALPPSWAAGAPRAGRRPARPRGCADRPEELLEQLYGRLAAGVLSAFHHTLQLGPREQARNASCPAGGRPADRRFRPPTNLRSVSPWAYRISYDPARYPRYLPEAYCLCRGCLTGLFGEEDVRFRSAPVYMPTVVLRRTPACAGGRSVYTEAYVTIPVGCTCVPEPEKDADSINSSIDKQGAKLLLGPNDAPAGP

SEQ ID NO: 37 - protein, 177 aa, Homo sapiens
MRERPRLGEDSSLISLFLQVVAFLAMVMGTHTYSHWPSCCPSKGQDTSEELLRWSTVPVPPLEPARPNRHPESCRASEDGPLNSRAISPWRYELDRDLNRLPQDLYHARCLCPHCVSLQTGSHMDPRGNSELLYHNQTVFYRRPCHGEKGTHKGYCLERRLYRVSLACVCVRPRVMG

SEQ ID NO: 38 - protein, 163 aa, Homo sapiens
MTVKTLHGPAMVKYLLLSILGLAFLSEAAARKIPKVGHTFFQKPESCPPVPGGSMKLDIGIINENQRVSMSRNIESRSTSPWNYTVTWDPNRYPSEVVQAQCRNLGCINAQGKEDISMNSVPIQQETLVVRRKHQGCSVSFQLEKVLVTVGCTCVTPVIHHVQ

SEQ ID NO: 39 - protein, 11 aa, synthetic construct
  REGION 1..11: note = artificial antibody-related sequence
GFSFSGFYYMC

SEQ ID NO: 40 - protein, 17 aa, synthetic construct
  REGION 1..17: note = artificial antibody-related sequence
CIDTGDGTTYYASWAKG

SEQ ID NO: 41 - protein, 17 aa, synthetic construct
  REGION 1..17: note = artificial antibody-related sequence
RDAAYGGYAYPAHGMDL

SEQ ID NO: 42 - protein, 6 aa, synthetic construct
  REGION 1..6: note = artificial antibody-related sequence
GFYYMC

SEQ ID NO: 43 - protein, 17 aa, synthetic construct
  REGION 1..17: note = artificial antibody-related sequence
CIDTGDGTTYYASWAKG

SEQ ID NO: 44 - protein, 16 aa, synthetic construct
  REGION 1..16: note = artificial antibody-related sequence
DAAYGGYAYPAHGMDL

SEQ ID NO: 45 - protein, 8 aa, synthetic construct
  REGION 1..8: note = artificial antibody-related sequence
GFSFSGFY

SEQ ID NO: 46 - protein, 4 aa, synthetic construct
  REGION 1..4: note = artificial antibody-related sequence
TGDG

SEQ ID NO: 47 - protein, 14 aa, synthetic construct
  REGION 1..14: note = artificial antibody-related sequence
AAYGGYAYPAHGMD

SEQ ID NO: 48 - protein, 126 aa, synthetic construct
  REGION 1..126: note = artificial antibody-related sequence
EVQLVESGGGLVQPGGSLRLSCAASGFSFSGFYYMCWVRQAPGKGLEWIGCIDTGDGTTYYASWAKGRFTISRDNSKNTVYLQMNSLRAEDTAVYYCARDAAYGGYAYPAHGMDLWGQGTLVTVSS

SEQ ID NO: 49 - protein, 126 aa, synthetic construct
  REGION 1..126: note = artificial antibody-related sequence
EVQLVESGGGLVQPGGSLTLSCAASGFSFSGFYYMCWVRQAPGKGLEWIGCIDTGDGTTYYASWAKGRFTISRDNSKNTVYLQMNSLRAEDTAVYYCARDAAYGGYAYPAHGMDLWGPGTLVTVSS

SEQ ID NO: 50 - protein, 11 aa, synthetic construct
  REGION 1..11: note = artificial antibody-related sequence
QASESIYRYLS

SEQ ID NO: 51 - protein, 7 aa, synthetic construct
  REGION 1..7: note = artificial antibody-related sequence
LASTLTS

SEQ ID NO: 52 - protein, 14 aa, synthetic construct
  REGION 1..14: note = artificial antibody-related sequence
QSNFGTASTTYYNT

SEQ ID NO: 53 - protein, 11 aa, synthetic construct
  REGION 1..11: note = artificial antibody-related sequence
QASESIYRYLS

SEQ ID NO: 54 - protein, 7 aa, synthetic construct
  REGION 1..7: note = artificial antibody-related sequence
LASTLTS

SEQ ID NO: 55 - protein, 14 aa, synthetic construct
  REGION 1..14: note = artificial antibody-related sequence
QSNFGTASTTYYNT

SEQ ID NO: 56 - protein, 7 aa, synthetic construct
  REGION 1..7: note = artificial antibody-related sequence
SESIYRY

SEQ ID NO: 57 - skipped

SEQ ID NO: 58 - protein, 11 aa, synthetic construct
  REGION 1..11: note = artificial antibody-related sequence
NFGTASTTYYN

SEQ ID NO: 59 - protein, 113 aa, synthetic construct
  REGION 1..113: note = artificial antibody-related sequence
DIQMTQSPSSLSASVGDRVTITCQASESIYRYLSWYQQKPGKAPKLLIYLASTLTSGVPSRFSGSGSGTDFTLTISSLQPEDFATYYCQSNFGTASTTYYNTFGGGTKLTVLG

SEQ ID NO: 60 - protein, 113 aa, synthetic construct; identical to SEQ ID NO: 59
  REGION 1..113: note = artificial antibody-related sequence

SEQ ID NO: 61 - protein, 259 aa, synthetic construct
  REGION 1..259: note = artificial antibody-related sequence
DIQMTQSPSSLSASVGDRVTITCQASESIYRYLSWYQQKPGKAPKLLIYLASTLTSGVPSRFSGSGSGTDFTLTISSLQPEDFATYYCQSNFGTASTTYYNTFGGGTKLTVLGGGGGSGGGGSGGGGSGGGGSEVQLVESGGGLVQPGGSLRLSCAASGFSFSGFYYMCWVRQAPGKGLEWIGCIDTGDGTTYYASWAKGRFTISRDNSKNTVYLQMNSLRAEDTAVYYCARDAAYGGYAYPAHGMDLWGQGTLVTVSS

SEQ ID NO: 62 - protein, 259 aa, synthetic construct
  REGION 1..259: note = artificial antibody-related sequence
DIQMTQSPSSLSASVGDRVTITCQASESIYRYLSWYQQKPGKAPKLLIYLASTLTSGVPSRFSGSGSGTDFTLTISSLQPEDFATYYCQSNFGTASTTYYNTFGGGTKLTVLGGGGGSGGGGSGGGGSGGGGSEVQLVESGGGLVQPGGSLTLSCAASGFSFSGFYYMCWVRQAPGKGLEWIGCIDTGDGTTYYASWAKGRFTISRDNSKNTVYLQMNSLRAEDTAVYYCARDAAYGGYAYPAHGMDLWGPGTLVTVSS

SEQ ID NO: 63 - protein, 10 aa, synthetic construct
  REGION 1..10: note = artificial antibody-related sequence
GIDFSTYGIS

SEQ ID NO: 64 - protein, 17 aa, synthetic construct
  REGION 1..17: note = artificial antibody-related sequence
YIYPDYGITDYASWVNG

SEQ ID NO: 65 - protein, 17 aa, synthetic construct
  REGION 1..17: note = artificial antibody-related sequence
RSGSYYSRGWGAHYFNL

SEQ ID NO: 66 - protein, 5 aa, synthetic construct
  REGION 1..5: note = artificial antibody-related sequence
TYGIS

SEQ ID NO: 67 - protein, 17 aa, synthetic construct
  REGION 1..17: note = artificial antibody-related sequence
YIYPDYGITDYASWVNG

SEQ ID NO: 68 - protein, 16 aa, synthetic construct
  REGION 1..16: note = artificial antibody-related sequence
SGSYYSRGWGAHYFNL

SEQ ID NO: 69 - protein, 7 aa, synthetic construct
  REGION 1..7: note = artificial antibody-related sequence
GIDFSTY

SEQ ID NO: 70 - protein, 4 aa, synthetic construct
  REGION 1..4: note = artificial antibody-related sequence
PDYG

SEQ ID NO: 71 - protein, 14 aa, synthetic construct
  REGION 1..14: note = artificial antibody-related sequence
GSYYSRGWGAHYFN

SEQ ID NO: 72 - protein, 125 aa, synthetic construct
  REGION 1..125: note = artificial antibody-related sequence
EVQLVESGGGLVQPGGSLRLSCAASGIDFSTYGISWVRQAPGKGLEWIAYIYPDYGITDYASWVNGRFTISLDNAQNTVYLQMNSLRAEDTAVYYCARSGSYYSRGWGAHYFNLWGQGTLVTVSS

SEQ ID NO: 73 - protein, 125 aa, synthetic construct
  REGION 1..125: note = artificial antibody-related sequence
EVQLVESGGGLVQPGGSLRLSCAASGIDFSTYGISWVRQAPGKGLEWIGYIYPDYGITDYASWVNGRFTISRDNSKNTVYLQMNSLRAEDTAVYYCARSGSYYSRGWGAHYFNLWGQGTLVTVSS

SEQ ID NO: 74 - protein, 125 aa, synthetic construct
  REGION 1..125: note = artificial antibody-related sequence
EVQLVESGGGLVQPGGSLRLSCKASGIDFSTYGISWVRQAPGKGLEWIAYIYPDYGITDYASWVNGRFTISLDNSKNTVYLQMNSLRAEDTAVYYCARSGSYYSRGWGAHYFNLWGQGTLVTVSS

SEQ ID NO: 75 - protein, 125 aa, synthetic construct; identical to SEQ ID NO: 72
  REGION 1..125: note = artificial antibody-related sequence

SEQ ID NO: 76 - protein, 11 aa, synthetic construct
  REGION 1..11: note = artificial antibody-related sequence
QASESISSWLA

SEQ ID NO: 77 - protein, 7 aa, synthetic construct
  REGION 1..7: note = artificial antibody-related sequence
KASTLAS

SEQ ID NO: 78 - protein, 13 aa, synthetic construct
  REGION 1..13: note = artificial antibody-related sequence
QGYYLDSSVDDNV

SEQ ID NO: 79 - protein, 11 aa, synthetic construct
  REGION 1..11: note = artificial antibody-related sequence
QASESISSWLA

SEQ ID NO: 80 - protein, 7 aa, synthetic construct
  REGION 1..7: note = artificial antibody-related sequence
KASTLAS

SEQ ID NO: 81 - protein, 13 aa, synthetic construct
  REGION 1..13: note = artificial antibody-related sequence
QGYYLDSSVDDNV

SEQ ID NO: 82 - protein, 7 aa, synthetic construct
  REGION 1..7: note = artificial antibody-related sequence
SESISSW

SEQ ID NO: 83 - skipped

SEQ ID NO: 84 - protein, 10 aa, synthetic construct
  REGION 1..10: note = artificial antibody-related sequence
YYLDSSVDDN

SEQ ID NO: 85 - protein, 112 aa, synthetic construct
  REGION 1..112: note = artificial antibody-related sequence
DIQMTQSPSSLSASVGDRVTINCQASESISSWLAWYQQKPGKRPKLLIYKASTLASGVPSRFSGSGSGTDYTLTISSLQPEDFATYYCQGYYLDSSVDDNVFGGGTKLTVLG

SEQ ID NO: 86 - protein, 112 aa, synthetic construct
  REGION 1..112: note = artificial antibody-related sequence
DIQMTQSPSSLSASVGDRVTITCQASESISSWLAWYQQKPGKAPKLLIYKASTLASGVPSRFSGSGSGTDFTLTISSLQPEDFATYYCQGYYLDSSVDDNVFGGGTKLTVLG

SEQ ID NO: 87 - protein, 112 aa, synthetic construct
  REGION 1..112: note = artificial antibody-related sequence
DIQMTQSPSSLSASVGDRVTINCQASESISSWLAWYQQKPGKAPKLLIYKASTLASGVPSRFSGSGSGTEFTLTISGLQPADFATYYCQGYYLDSSVDDNVFGGGTKLTVLG

SEQ ID NO: 88 - protein, 112 aa, synthetic construct
  REGION 1..112: note = artificial antibody-related sequence
DIQMTQSPSSLSASVGDRVTINCQASESISSWLAWYQQKPGKRPKLLIYKASTLASGVPSRFSGSGSGTDYTLTISGLQPEDFATYYCQGYYLDSSVDDNVFGTGTKVTVLG

SEQ ID NO: 89 - protein, 112 aa, synthetic construct
  REGION 1..112: note = artificial antibody-related sequence
DIQMTQSPSSLSASVGDRVTINCQASESISSWLAWYQQKPGQRPKLLIYKASTLASGVPSRFSGSGSGTDYTLTISSLQPEDFATYYCQGYYLDSSVDDNVFGTGTKVTVLG

SEQ ID NO: 90 - protein, 10 aa, synthetic construct
  REGION 1..10: note = artificial antibody-related sequence
GFSLSSNAMG

SEQ ID NO: 91 - protein, 16 aa, synthetic construct
  REGION 1..16: note = artificial antibody-related sequence
IISVGGFTYYASWAKG

SEQ ID NO: 92 - protein, 14 aa, synthetic construct
  REGION 1..14: note = artificial antibody-related sequence
RDRHGGDSSGAFYL

SEQ ID NO: 93 - protein, 5 aa, synthetic construct
  REGION 1..5: note = artificial antibody-related sequence
SNAMG

SEQ ID NO: 94 - protein, 16 aa, synthetic construct
  REGION 1..16: note = artificial antibody-related sequence
IISVGGFTYYASWAKG

SEQ ID NO: 95 - protein, 13 aa, synthetic construct
  REGION 1..13: note = artificial antibody-related sequence
DRHGGDSSGAFYL

SEQ ID NO: 96 - protein, 7 aa, synthetic construct
  REGION 1..7: note = artificial antibody-related sequence
GFSLSSN

SEQ ID NO: 97 - skipped

SEQ ID NO: 98 - protein, 11 aa, synthetic construct
  REGION 1..11: note = artificial antibody-related sequence
RHGGDSSGAFY

SEQ ID NO: 99 - protein, 121 aa, synthetic construct
  REGION 1..121: note = artificial antibody-related sequence
EVQLVESGGGLVQPGGSLRLSCAASGFSLSSNAMGWVRQAPGKGLEYIGIISVGGFTYYASWAKGRFTISRDNSKNTVYLQMNSLRAEDTATYFCARDRHGGDSSGAFYLWGQGTLVTVSS

SEQ ID NO: 100 - protein, 13 aa, synthetic construct
  REGION 1..13: note = artificial antibody-related sequence
QSSESVYSNNQLS

SEQ ID NO: 101 - protein, 7 aa, synthetic construct
  REGION 1..7: note = artificial antibody-related sequence
DASDLAS

SEQ ID NO: 102 - protein, 11 aa, synthetic construct
  REGION 1..11: note = artificial antibody-related sequence
AGGFSSSSDTA

SEQ ID NO: 103 - protein, 13 aa, synthetic construct
  REGION 1..13: note = artificial antibody-related sequence
QSSESVYSNNQLS

SEQ ID NO: 104 - protein, 7 aa, synthetic construct
  REGION 1..7: note = artificial antibody-related sequence
DASDLAS

SEQ ID NO: 105 - protein, 11 aa, synthetic construct
  REGION 1..11: note = artificial antibody-related sequence
AGGFSSSSDTA

SEQ ID NO: 106 - protein, 9 aa, synthetic construct
  REGION 1..9: note = artificial antibody-related sequence
SESVYSNNQ

SEQ ID NO: 107 - skipped

SEQ ID NO: 108 - protein, 8 aa, synthetic construct
  REGION 1..8: note = artificial antibody-related sequence
GFSSSSDT

SEQ ID NO: 109 - protein, 112 aa, synthetic construct
  REGION 1..112: note = artificial antibody-related sequence
DIQMTQSPSSLSASVGDRVTITCQSSESVYSNNQLSWYQQKPGQPPKLLIYDASDLASGVPSRFSGSGSGTDFTLTISSLQPEDFATYYCAGGFSSSSDTAFGGGTKLTVLG

SEQ ID NO: 110 - protein, 253 aa, synthetic construct
  REGION 1..253: note = artificial antibody-related sequence
DIQMTQSPSSLSASVGDRVTITCQSSESVYSNNQLSWYQQKPGQPPKLLIYDASDLASGVPSRFSGSGSGTDFTLTISSLQPEDFATYYCAGGFSSSSDTAFGGGTKLTVLGGGGGSGGGGSGGGGSGGGGSEVQLVESGGGLVQPGGSLRLSCAASGFSLSSNAMGWVRQAPGKGLEYIGIISVGGFTYYASWAKGRFTISRDNSKNTVYLQMNSLRAEDTATYFCARDRHGGDSSGAFYLWGQGTLVTVSS

SEQ ID NO: 111 - protein, 11 aa, synthetic construct
  REGION 1..11: note = artificial antibody-related sequence
GFSFSSSYWIC

SEQ ID NO: 112 - protein, 17 aa, synthetic construct
  REGION 1..17: note = artificial antibody-related sequence
CVFTGDGTTYYASWAKG

SEQ ID NO: 113 - protein, 12 aa, synthetic construct
  REGION 1..12: note = artificial antibody-related sequence
RPVSVYYYGMDL

SEQ ID NO: 114 - protein, 6 aa, synthetic construct
  REGION 1..6: note = artificial antibody-related sequence
SSYWIC

SEQ ID NO: 115 - protein, 17 aa, synthetic construct
  REGION 1..17: note = artificial antibody-related sequence
CVFTGDGTTYYASWAKG

SEQ ID NO: 116 - protein, 11 aa, synthetic construct
  REGION 1..11: note = artificial antibody-related sequence
PVSVYYYGMDL

SEQ ID NO: 117 - protein, 8 aa, synthetic construct
  REGION 1..8: note = artificial antibody-related sequence
GFSFSSSY

SEQ ID NO: 118 - protein, 4 aa, synthetic construct
  REGION 1..4: note = artificial antibody-related sequence
TGDG

SEQ ID NO: 119 - protein, 9 aa, synthetic construct
  REGION 1..9: note = artificial antibody-related sequence
VSVYYYGMD

SEQ ID NO: 120 - protein, 121 aa, synthetic construct
  REGION 1..121: note = artificial antibody-related sequence
EVQLVESGGGLVQPGGSLRLSCAASGFSFSSSYWICWVRQAPGKGLEWVGCVFTGDGTTYYASWAKGRFTISRDNSKNTVYLQMNSLRAEDTATYFCARPVSVYYYGMDLWGQGTLVTVSS

SEQ ID NO: 121 - protein, 11 aa, synthetic construct
  REGION 1..11: note = artificial antibody-related sequence
QASQIISSRSA

SEQ ID NO: 122 - protein, 7 aa, synthetic construct
  REGION 1..7: note = artificial antibody-related sequence
QASKLAS

SEQ ID NO: 123 - protein, 11 aa, synthetic construct
  REGION 1..11: note = artificial antibody-related sequence
QCTYIDSNFGA

SEQ ID NO: 124 - protein, 11 aa, synthetic construct
  REGION 1..11: note = artificial antibody-related sequence
QASQIISSRSA

SEQ ID NO: 125 - protein, 7 aa, synthetic construct
  REGION 1..7: note = artificial antibody-related sequence
QASKLAS

SEQ ID NO: 126 - protein, 11 aa, synthetic construct
  REGION 1..11: note = artificial antibody-related sequence
QCTYIDSNFGA

SEQ ID NO: 127 - protein, 7 aa, synthetic construct
  REGION 1..7: note = artificial antibody-related sequence
SQIISSR

SEQ ID NO: 128 - skipped

SEQ ID NO: 129 - protein, 8 aa, synthetic construct
  REGION 1..8: note = artificial antibody-related sequence
TYIDSNFG

SEQ ID NO: 130 - protein, 110 aa, synthetic construct
  REGION 1..110: note = artificial antibody-related sequence
DVVMTQSPSSLSASVGDRVTITCQASQIISSRSAWYQQKPGQPPKLLIYQASKLASGVPSRFSGSGSGTDFTLTISSLQPEDFATYYCQCTYIDSNFGAFGGGTKLTVLG

SEQ ID NO: 131 - protein, 251 aa, synthetic construct
  REGION 1..251: note = artificial antibody-related sequence
DVVMTQSPSSLSASVGDRVTITCQASQIISSRSAWYQQKPGQPPKLLIYQASKLASGVPSRFSGSGSGTDFTLTISSLQPEDFATYYCQCTYIDSNFGAFGGGTKLTVLGGGGGSGGGGSGGGGSGGGGSEVQLVESGGGLVQPGGSLRLSCAASGFSFSSSYWICWVRQAPGKGLEWVGCVFTGDGTTYYASWAKGRFTISRDNSKNTVYLQMNSLRAEDTATYFCARPVSVYYYGMDLWGQGTLVTVSS

SEQ ID NO: 132 - protein, 5 aa, synthetic construct
  REGION 1..5: note = artificial antibody-related sequence
GGGGS

SEQ ID NO: 133 - skipped

SEQ ID NO: 134 - protein, 233 aa, Homo sapiens
MSTESMIRDVELAEEALPKKTGGPQGSRRCLFLSLFSFLIVAGATTLFCLLHFGVIGPQREEFPRDLSLISPLAQAVRSSSRTPSDKPVAHVVANPQAEGQLQWLNRRANALLANGVELRDNQLVVPSEGLYLIYSQVLFKGQGCPSTHVLLTHTISRIAVSYQTKVNLLSAIKSPCQRETPEGAEAKPWYEPIYLGGVFQLEKGDRLSAEINRPDYLDFAESGQVYFGIIAL

SEQ ID NO: 135 - protein, 157 aa, Homo sapiens [sequence omitted]

SEQ ID NO: 136 - protein, 488 aa, synthetic construct
  REGION 1..488: note = artificial antibody-related sequence
DIQMTQSPSSLSASVGDRVTITCQSSESVYSNNQLSWYQQKPGQPPKLLIYDASDLASGVPSRFSGSGSGTDFTLTISSLQPEDFATYYCAGGFSSSSDTAFGGGTKLTVLGRTRTVAAPSVFIFPPSDEQLKSGTASVVCLLNNFYPREAKVQWKVDNALQSGNSQESVTEQDSKDSTYSLSSTLTLSKADYEKHKVYACEVTHQGLSSPVTKSFNRGECGGGGSGGGGSDIQMTQSPSSLSASVGDRVTINCQASESISSWLAWYQQKPGKRPKLLIYKASTLASGVPSRFSGSGSGTDYTLTISSLQPEDFATYYCQGYYLDSSVDDNVFGGGTKLTVLGGGGGSGGGGSGGGGSGGGGSEVQLVESGGGLVQPGGSLRLSCAASGIDFSTYGISWVRQAPGKGLEWIAYIYPDYGITDYASWVNGRFTISLDNAQNTVYLQMNSLRAEDTAVYYCARSGSYYSRGWGAHYFNLWGQGTLVTVSS

SEQ ID NO: 137 - protein, 487 aa, synthetic construct
  REGION 1..487: note = artificial antibody-related sequence
EVQLVESGGGLVQPGGSLRLSCAASGFSLSSNAMGWVRQAPGKGLEYIGIISVGGFTYYASWAKGRFTISRDNSKNTVYLQMNSLRAEDTATYFCARDRHGGDSSGAFYLWGQGTLVTVSSASTKGPSVFPLAPSSKSTSGGTAALGCLVKDYFPEPVTVSWNSGALTSGVHTFPAVLQSSGLYSLSSVVTVPSSSLGTQTYICNVNHKPSNTKVDKKVEPKSCGGGGSGGGGSDIQMTQSPSSLSASVGDRVTITCQASQTINYWLAWYQQKPGKAPKLLIYRASTLASGVPSRFSGSGSGTDFTLTISSLQPEDFATYYCQNYYYSTSRSYGFGGGTKLTVLGGGGGSGGGGSGGGGSGGGGSEVQLVESGGGLVQPGGSLRLSCAASGFSFSSDYWMCWVRQAPGKGLEWIGCIYAGDVDDTDYASWARGRFTISRDNSKNTVYLQMNSLRAEDTAVYYCARVDGFDITYFDLWGQGTLVTVSS

SEQ ID NO: 138 - protein, 487 aa, synthetic construct
  REGION 1..487: note = artificial antibody-related sequence
DIQMTQSPSSLSASVGDRVTITCQASQTINYWLAWYQQKPGKAPKLLIYRASTLASGVPSRFSGSGSGTDFTLTISSLQPEDFATYYCQNYYYSTSRSYGFGGGTKLTVLGRTRTVAAPSVFIFPPSDEQLKSGTASVVCLLNNFYPREAKVQWKVDNALQSGNSQESVTEQDSKDSTYSLSSTLTLSKADYEKHKVYACEVTHQGLSSPVTKSFNRGECGGGGSGGGGSDIQMTQSPSSLSASVGDRVTINCQASESISSWLAWYQQKPGKRPKLLIYKASTLASGVPSRFSGSGSGTDYTLTISSLQPEDFATYYCQGYYLDSSVDDNVFGGGTKLTVLGGGGGSGGGGSGGGGSGGGGSEVQLVESGGGLVQPGGSLRLSCAASGIDFSTYGISWVRQAPGKGLEWIAYIYPDYGITDYASWVNGRFTISLDNAQNTVYLQMNSLRAEDTAVYYCARSGSYYSRGWGAHYFNLWGQGTLVTVSS

SEQ ID NO: 139 - protein, 488 aa, synthetic construct
  REGION 1..488: note = artificial antibody-related sequence
EVQLVESGGGLVQPGGSLRLSCAASGFSFSSDYWMCWVRQAPGKGLEWIGCIYAGDVDDTDYASWARGRFTISRDNSKNTVYLQMNSLRAEDTAVYYCARVDGFDITYFDLWGQGTLVTVSSASTKGPSVFPLAPSSKSTSGGTAALGCLVKDYFPEPVTVSWNSGALTSGVHTFPAVLQSSGLYSLSSVVTVPSSSLGTQTYICNVNHKPSNTKVDKKVEPKSCGGGGSGGGGSDIQMTQSPSSLSASVGDRVTITCQSSESVYSNNQLSWYQQKPGQPPKLLIYDASDLASGVPSRFSGSGSGTDFTLTISSLQPEDFATYYCAGGFSSSSDTAFGGGTKLTVLGGGGGSGGGGSGGGGSGGGGSEVQLVESGGGLVQPGGSLRLSCAASGFSLSSNAMGWVRQAPGKGLEYIGIISVGGFTYYASWAKGRFTISRDNSKNTVYLQMNSLRAEDTATYFCARDRHGGDSSGAFYLWGQGTLVTVSS

SEQ ID NO: 140 - protein, 484 aa, synthetic construct
  REGION 1..484: note = artificial antibody-related sequence
DIQMTQSPSSLSASVGDRVTINCQASESISSWLAWYQQKPGKRPKLLIYKASTLASGVPSRFSGSGSGTDYTLTISSLQPEDFATYYCQGYYLDSSVDDNVFGGGTKLTVLGRTRTVAAPSVFIFPPSDEQLKSGTASVVCLLNNFYPREAKVQWKVDNALQSGNSQESVTEQDSKDSTYSLSSTLTLSKADYEKHKVYACEVTHQGLSSPVTKSFNRGECGGGGSGGGGSDIQMTQSPSSLSASVGDRVTITCQSSESVYSNNQLSWYQQKPGQPPKLLIYDASDLASGVPSRFSGSGSGTDFTLTISSLQPEDFATYYCAGGFSSSSDTAFGGGTKLTVLGGGGGSGGGGSGGGGSGGGGSEVQLVESGGGLVQPGGSLRLSCAASGFSLSSNAMGWVRQAPGKGLEYIGIISVGGFTYYASWAKGRFTISRDNSKNTVYLQMNSLRAEDTATYFCARDRHGGDSSGAFYLWGQGTLVTVSS

SEQ ID NO: 141 - protein, 491 aa, synthetic construct
  REGION 1..491: note = artificial antibody-related sequence
EVQLVESGGGLVQPGGSLRLSCAASGIDFSTYGISWVRQAPGKGLEWIAYIYPDYGITDYASWVNGRFTISLDNAQNTVYLQMNSLRAEDTAVYYCARSGSYYSRGWGAHYFNLWGQGTLVTVSSASTKGPSVFPLAPSSKSTSGGTAALGCLVKDYFPEPVTVSWNSGALTSGVHTFPAVLQSSGLYSLSSVVTVPSSSLGTQTYICNVNHKPSNTKVDKKVEPKSCGGGGSGGGGSDIQMTQSPSSLSASVGDRVTITCQASQTINYWLAWYQQKPGKAPKLLIYRASTLASGVPSRFSGSGSGTDFTLTISSLQPEDFATYYCQNYYYSTSRSYGFGGGTKLTVLGGGGGSGGGGSGGGGSGGGGSEVQLVESGGGLVQPGGSLRLSCAASGFSFSSDYWMCWVRQAPGKGLEWIGCIYAGDVDDTDYASWARGRFTISRDNSKNTVYLQMNSLRAEDTAVYYCARVDGFDITYFDLWGQGTLVTVSS

SEQ ID NO: 142 - protein, 763 aa, synthetic construct
  REGION 1..763: note = artificial antibody-related sequence
DIQMTQSPSSLSASVGDRVTITCQASQTINYWLAWYQQKPGKAPKLLIYRASTLASGVPSRFSGSGSGTDFTLTISSLQPEDFATYYCQNYYYSTSRSYGFGGGTKLTVLGGGGGSEVQLVESGGGLVQPGGSLRLSCAASGFSLSSNAMGWVRQAPGKGLEYIGIISVGGFTYYASWAKGRFTISRDNSKNTVYLQMNSLRAEDTATYFCARDRHGGDSSGAFYLWGQGTLVTVSSGGGGSGGGGSGGGGSGGGGSDIQMTQSPSSLSASVGDRVTITCQSSESVYSNNQLSWYQQKPGQPPKLLIYDASDLASGVPSRFSGSGSGTDFTLTISSLQPEDFATYYCAGGFSSSSDTAFGGGTKLTVLGGGGGSEVQLVESGGGLVQPGGSLRLSCAASGFSFSSDYWMCWVRQAPGKGLEWIGCIYAGDVDDTDYASWARGRFTISRDNSKNTVYLQMNSLRAEDTAVYYCARVDGFDITYFDLWGQGTLVTVSSGGGGSGGGGSDIQMTQSPSSLSASVGDRVTINCQASESISSWLAWYQQKPGKRPKLLIYKASTLASGVPSRFSGSGSGTDYTLTISSLQPEDFATYYCQGYYLDSSVDDNVFGGGTKLTVLGGGGGSGGGGSGGGGSGGGGSEVQLVESGGGLVQPGGSLRLSCAASGIDFSTYGISWVRQAPGKGLEWIAYIYPDYGITDYASWVNGRFTISLDNAQNTVYLQMNSLRAEDTAVYYCARSGSYYSRGWGAHYFNLWGQGTLVTVSS

SEQ ID NO: 143 - protein, 763 aa, synthetic construct
  REGION 1..763: note = artificial antibody-related sequence
DIQMTQSPSSLSASVGDRVTINCQASESISSWLAWYQQKPGKRPKLLIYKASTLASGVPSRFSGSGSGTDYTLTISSLQPEDFATYYCQGYYLDSSVDDNVFGGGTKLTVLGGGGGSEVQLVESGGGLVQPGGSLRLSCAASGFSFSSDYWMCWVRQAPGKGLEWIGCIYAGDVDDTDYASWARGRFTISRDNSKNTVYLQMNSLRAEDTAVYYCARVDGFDITYFDLWGQGTLVTVSSGGGGSGGGGSGGGGSGGGGSDIQMTQSPSSLSASVGDRVTITCQASQTINYWLAWYQQKPGKAPKLLIYRASTLASGVPSRFSGSGSGTDFTLTISSLQPEDFATYYCQNYYYSTSRSYGFGGGTKLTVLGGGGGSEVQLVESGGGLVQPGGSLRLSCAASGIDFSTYGISWVRQAPGKGLEWIAYIYPDYGITDYASWVNGRFTISLDNAQNTVYLQMNSLRAEDTAVYYCARSGSYYSRGWGAHYFNLWGQGTLVTVSSGGGGSGGGGSDIQMTQSPSSLSASVGDRVTITCQSSESVYSNNQLSWYQQKPGQPPKLLIYDASDLASGVPSRFSGSGSGTDFTLTISSLQPEDFATYYCAGGFSSSSDTAFGGGTKLTVLGGGGGSGGGGSGGGGSGGGGSEVQLVESGGGLVQPGGSLRLSCAASGFSLSSNAMGWVRQAPGKGLEYIGIISVGGFTYYASWAKGRFTISRDNSKNTVYLQMNSLRAEDTATYFCARDRHGGDSSGAFYLWGQGTLVTVSS

SEQ ID NO: 144 - protein, 763 aa, synthetic construct
  REGION 1..763: note = artificial antibody-related sequence
DIQMTQSPSSLSASVGDRVTITCQSSESVYSNNQLSWYQQKPGQPPKLLIYDASDLASGVPSRFSGSGSGTDFTLTISSLQPEDFATYYCAGGFSSSSDTAFGGGTKLTVLGGGGGSEVQLVESGGGLVQPGGSLRLSCAASGIDFSTYGISWVRQAPGKGLEWIAYIYPDYGITDYASWVNGRFTISLDNAQNTVYLQMNSLRAEDTAVYYCARSGSYYSRGWGAHYFNLWGQGTLVTVSSGGGGSGGGGSGGGGSGGGGSDIQMTQSPSSLSASVGDRVTINCQASESISSWLAWYQQKPGKRPKLLIYKASTLASGVPSRFSGSGSGTDYTLTISSLQPEDFATYYCQGYYLDSSVDDNVFGGGTKLTVLGGGGGSEVQLVESGGGLVQPGGSLRLSCAASGFSLSSNAMGWVRQAPGKGLEYIGIISVGGFTYYASWAKGRFTISRDNSKNTVYLQMNSLRAEDTATYFCARDRHGGDSSGAFYLWGQGTLVTVSSGGGGSGGGGSDIQMTQSPSSLSASVGDRVTITCQASQTINYWLAWYQQKPGKAPKLLIYRASTLASGVPSRFSGSGSGTDFTLTISSLQPEDFATYYCQNYYYSTSRSYGFGGGTKLTVLGGGGGSGGGGSGGGGSGGGGSEVQLVESGGGLVQPGGSLRLSCAASGFSFSSDYWMCWVRQAPGKGLEWIGCIYAGDVDDTDYASWARGRFTISRDNSKNTVYLQMNSLRAEDTAVYYCARVDGFDITYFDLWGQGTLVTVSS

SEQ ID NO: 145 - protein, 763 aa, synthetic construct
  REGION 1..763: note = artificial antibody-related sequence
DIQMTQSPSSLSASVGDRVTINCQASESISSWLAWYQQKPGKRPKLLIYKASTLASGVPSRFSGSGSGTDYTLTISGLQPEDFATYYCQGYYLDSSVDDNVFGTGTKVTVLGGGGGSEVQLVESGGGLVQPGGSLRLSCAASGFSFSSDYWMCWVRQAPGKGLEWIGCIYAGDVDDTDYASWARGRFTISRDNSKNTVYLQMNSLRAEDTAVYYCARVDGFDITYFDLWGQGTLVTVSSGGGGSGGGGSGGGGSGGGGSDIQMTQSPSSLSASVGDRVTITCQASQTINYWLAWYQQKPGKAPKLLIYRASTLASGVPSRFSGSGSGTDFTLTISSLQPEDFATYYCQNYYYSTSRSYGFGGGTKLTVLGGGGGSEVQLVESGGGLVQPGGSLRLSCAASGIDFSTYGISWVRQAPGKGLEWIAYIYPDYGITDYASWVNGRFTISLDNAQNTVYLQMNSLRAEDTAVYYCARSGSYYSRGWGAHYFNLWGQGTLVTVSSGGGGSGGGGSDIQMTQSPSSLSASVGDRVTITCQSSESVYSNNQLSWYQQKPGQPPKLLIYDASDLASGVPSRFSGSGSGTDFTLTISSLQPEDFATYYCAGGFSSSSDTAFGGGTKLTVLGGGGGSGGGGSGGGGSGGGGSEVQLVESGGGLVQPGGSLRLSCAASGFSLSSNAMGWVRQAPGKGLEYIGIISVGGFTYYASWAKGRFTISRDNSKNTVYLQMNSLRAEDTATYFCARDRHGGDSSGAFYLWGQGTLVTVSS

SEQ ID NO: 146 - protein, 763 aa, synthetic construct
  REGION 1..763: note = artificial antibody-related sequence
DIQMTQSPSSLSASVGDRVTINCQASESISSWLAWYQQKPGQRPKLLIYKASTLASGVPSRFSGSGSGTDYTLTISSLQPEDFATYYCQGYYLDSSVDDNVFGTGTKVTVLGGGGGSEVQLVESGGGLVQPGGSLRLSCAASGFSFSSDYWMCWVRQAPGKGLEWIGCIYAGDVDDTDYASWARGRFTISRDNSKNTVYLQMNSLRAEDTAVYYCARVDGFDITYFDLWGQGTLVTVSSGGGGSGGGGSGGGGSGGGGSDIQMTQSPSSLSASVGDRVTITCQASQTINYWLAWYQQKPGKAPKLLIYRASTLASGVPSRFSGSGSGTDFTLTISSLQPEDFATYYCQNYYYSTSRSYGFGGGTKLTVLGGGGGSEVQLVESGGGLVQPGGSLRLSCAASGIDFSTYGISWVRQAPGKGLEWIAYIYPDYGITDYASWVNGRFTISLDNAQNTVYLQMNSLRAEDTAVYYCARSGSYYSRGWGAHYFNLWGQGTLVTVSSGGGGSGGGGSDIQMTQSPSSLSASVGDRVTITCQSSESVYSNNQLSWYQQKPGQPPKLLIYDASDLASGVPSRFSGSGSGTDFTLTISSLQPEDFATYYCAGGFSSSSDTAFGGGTKLTVLGGGGGSGGGGSGGGGSGGGGSEVQLVESGGGLVQPGGSLRLSCAASGFSLSSNAMGWVRQAPGKGLEYIGIISVGGFTYYASWAKGRFTISRDNSKNTVYLQMNSLRAEDTATYFCARDRHGGDSSGAFYLWGQGTLVTVSS

SEQ ID NO: 147 - protein, 761 aa, synthetic construct
  REGION 1..761: note = artificial antibody-related sequence
DIQMTQSPSSLSASVGDRVTINCQASESISSWLAWYQQKPGKRPKLLIYKASTLASGVPSRFSGSGSGTDYTLTISGLQPEDFATYYCQGYYLDSSVDDNVFGTGTKVTVLGGGGGSEVQLVESGGGLVQPGGSLRLSCAASGFSFSSDYWMCWVRQAPGKGLEWIGCIYAGDVDDTDYASWARGRFTISRDNSKNTVYLQMNSLRAEDTAVYYCARVDGFDITYFDLWGQGTLVTVSSGGGGSGGGGSGGGGSGGGGSIQMTQSPSSLSASVGDRVTITCQASQTINYWLAWYQQKPGKAPKLLIYRASTLASGVPSRFSGSGSGTDFTLTISSLQPEDFATYYCQNYYYSTSRSYGFGGGTKLTVLGGGGGSEVQLVESGGGLVQPGGSLRLSCAASGIDFSTYGISWVRQAPGKGLEWIAYIYPDYGITDYASWVNGRFTISLDNAQNTVYLQMNSLRAEDTAVYYCARSGSYYSRGWGAHYFNLWGQGTLVTVSSGGGGSGGGGSIQMTQSPSSLSASVGDRVTITCQSSESVYSNNQLSWYQQKPGQPPKLLIYDASDLASGVPSRFSGSGSGTDFTLTISSLQPEDFATYYCAGGFSSSSDTAFGGGTKLTVLGGGGGSGGGGSGGGGSGGGGSEVQLVESGGGLVQPGGSLRLSCAASGFSLSSNAMGWVRQAPGKGLEYIGIISVGGFTYYASWAKGRFTISRDNSKNTVYLQMNSLRAEDTATYFCARDRHGGDSSGAFYLWGQGTLVTVSS

SEQ ID NO: 148 - protein, 761 aa, synthetic construct
  REGION 1..761: note = artificial antibody-related sequence
DIQMTQSPSSLSASVGDRVTINCQASESISSWLAWYQQKPGQRPKLLIYKASTLASGVPSRFSGSGSGTDYTLTISSLQPEDFATYYCQGYYLDSSVDDNVFGTGTKVTVLGGGGGSEVQLVESGGGLVQPGGSLRLSCAASGFSFSSDYWMCWVRQAPGKGLEWIGCIYAGDVDDTDYASWARGRFTISRDNSKNTVYLQMNSLRAEDTAVYYCARVDGFDITYFDLWGQGTLVTVSSGGGGSGGGGSGGGGSGGGGSIQMTQSPSSLSASVGDRVTITCQASQTINYWLAWYQQKPGKAPKLLIYRASTLASGVPSRFSGSGSGTDFTLTISSLQPEDFATYYCQNYYYSTSRSYGFGGGTKLTVLGGGGGSEVQLVESGGGLVQPGGSLRLSCAASGIDFSTYGISWVRQAPGKGLEWIAYIYPDYGITDYASWVNGRFTISLDNAQNTVYLQMNSLRAEDTAVYYCARSGSYYSRGWGAHYFNLWGQGTLVTVSSGGGGSGGGGSIQMTQSPSSLSASVGDRVTITCQSSESVYSNNQLSWYQQKPGQPPKLLIYDASDLASGVPSRFSGSGSGTDFTLTISSLQPEDFATYYCAGGFSSSSDTAFGGGTKLTVLGGGGGSGGGGSGGGGSGGGGSEVQLVESGGGLVQPGGSLRLSCAASGFSLSSNAMGWVRQAPGKGLEYIGIISVGGFTYYASWAKGRFTISRDNSKNTVYLQMNSLRAEDTATYFCARDRHGGDSSGAFYLWGQGTLVTVSS

SEQ ID NO: 149 - protein, 500 aa, synthetic construct
  REGION 1..500: note = artificial antibody-related sequence
DIQMTQSPSSLSASVGDRVTINCQASESISSWLAWYQQKPGKRPKLLIYKASTLASGVPSRFSGSGSGTDYTLTISSLQPEDFATYYCQGYYLDSSVDDNVFGGGTKLTVLGGGGGSEVQLVESGGGLVQPGGSLRLSCAASGFSLSSNAMGWVRQAPGKGLEYIGIISVGGFTYYASWAKGRFTISRDNSKNTVYLQMNSLRAEDTATYFCARDRHGGDSSGAFYLWGQGTLVTVSSGGGGSGGGGSGGGGSGGGGSDIQMTQSPSSLSASVGDRVTITCQSSESVYSNNQLSWYQQKPGQPPKLLIYDASDLASGVPSRFSGSGSGTDFTLTISSLQPEDFATYYCAGGFSSSSDTAFGGGTKLTVLGGGGGSEVQLVESGGGLVQPGGSLRLSCAASGIDFSTYGISWVRQAPGKGLEWIAYIYPDYGITDYASWVNGRFTISLDNAQNTVYLQMNSLRAEDTAVYYCARSGSYYSRGWGAHYFNLWGQGTLVTVSS